European Patent Application EP 4 455 284 A1, published October 30, 2024. Title: 一种核酸、含有该核酸的组合物与缀合物及制备方法和用途. Applicant: 苏州瑞博生物技术股份有限公司. The sequence listing filed with the application follows.

SEQUENCE LISTING (384 sequences)

SEQ ID NO: 1 - RNA, 19 nt, synthetic construct
  source 1..19: mol_type = other RNA
ctgccatggagtatctgaa

SEQ ID NO: 2 - RNA, 19 nt, synthetic construct
  source 1..19: mol_type = other RNA
ttcagatactccatggcag

SEQ ID NO: 3 - RNA, 19 nt, synthetic construct
  source 1..19: mol_type = other RNA
ctgccatggagtatctgan

SEQ ID NO: 4 - RNA, 19 nt, synthetic construct
  source 1..19: mol_type = other RNA
ntcagatactccatggcag

SEQ ID NO: 5 - RNA, 19 nt, synthetic construct
  source 1..19: mol_type = other RNA
ctgccatggagtatctgan

SEQ ID NO: 6 - RNA, 21 nt, synthetic construct
  source 1..21: mol_type = other RNA
ntcagatactccatggcagtg

SEQ ID NO: 7 - RNA, 21 nt, synthetic construct
  source 1..21: mol_type = other RNA
cactgccatggagtatctgan

SEQ ID NO: 8 - RNA, 23 nt, synthetic construct
  source 1..23: mol_type = other RNA
ntcagatactccatggcagtgac

SEQ ID NO: 9 - RNA, 19 nt, synthetic construct
  source 1..19: mol_type = other RNA
ctgccatggagtatctgaa

SEQ ID NO: 10 - RNA, 21 nt, synthetic construct
  source 1..21: mol_type = other RNA
ttcagatactccatggcagtg

SEQ ID NO: 11 - RNA, 21 nt, synthetic construct
  source 1..21: mol_type = other RNA
ctgccatggagtatctgaacg

SEQ ID NO: 12 - RNA, 21 nt, synthetic construct
  source 1..21: mol_type = other RNA
ttcagatactccatggcagtg

SEQ ID NO: 13 - RNA, 21 nt, synthetic construct
  source 1..21: mol_type = other RNA
cactgccatggagtatctgaa

SEQ ID NO: 14 - RNA, 23 nt, synthetic construct
  source 1..23: mol_type = other RNA
ttcagatactccatggcagtgac

SEQ ID NO: 15 - RNA, 19 nt, synthetic construct
  source 1..19: mol_type = other RNA
ctgccatggagtatctgaa

SEQ ID NO: 16 - RNA, 21 nt, synthetic construct
  source 1..21: mol_type = other RNA
ttcagatactccatggcagtg

SEQ ID NO: 17 - RNA, 19 nt, synthetic construct
  source 1..19: mol_type = other RNA
ctgccatggagtatctgaa

SEQ ID NO: 18 - RNA, 21 nt, synthetic construct
  source 1..21: mol_type = other RNA
ttcagatactccatggcagtg

SEQ ID NO: 19 - RNA, 19 nt, synthetic construct
  source 1..19: mol_type = other RNA
ctgccatggagtatctgaa

SEQ ID NO: 20 - RNA, 21 nt, synthetic construct
  source 1..21: mol_type = other RNA
ttcagatactccatggcagtg

SEQ ID NO: 21 - RNA, 21 nt, synthetic construct
  source 1..21: mol_type = other RNA
ctgccatggagtatctgaacg

SEQ ID NO: 22 - RNA, 21 nt, synthetic construct
  source 1..21: mol_type = other RNA
ttcagatactccatggcagtg

SEQ ID NO: 23 - RNA, 21 nt, synthetic construct
  source 1..21: mol_type = other RNA
ctgccatggagtatctgaacg

SEQ ID NO: 24 - RNA, 21 nt, synthetic construct
  source 1..21: mol_type = other RNA
ttcagatactccatggcagtg

SEQ ID NO: 25 - RNA, 21 nt, synthetic construct
  source 1..21: mol_type = other RNA
ctgccatggagtatctgaacg

SEQ ID NO: 26 - RNA, 21 nt, synthetic construct
  source 1..21: mol_type = other RNA
ttcagatactccatggcagtg

SEQ ID NO: 27 - RNA, 21 nt, synthetic construct
  source 1..21: mol_type = other RNA
cactgccatggagtatctgaa

SEQ ID NO: 28 - RNA, 23 nt, synthetic construct
  source 1..23: mol_type = other RNA
ttcagatactccatggcagtgac

SEQ ID NO: 29 - RNA, 21 nt, synthetic construct
  source 1..21: mol_type = other RNA
cactgccatggagtatctgaa

SEQ ID NO: 30 - RNA, 23 nt, synthetic construct
  source 1..23: mol_type = other RNA
ttcagatactccatggcagtgac

SEQ ID NO: 31 - RNA, 21 nt, synthetic construct
  source 1..21: mol_type = other RNA
cactgccatggagtatctgaa

SEQ ID NO: 32 - RNA, 23 nt, synthetic construct
  source 1..23: mol_type = other RNA
ttcagatactccatggcagtgac

SEQ ID NO: 33 - RNA, 19 nt, synthetic construct
  source 1..19: mol_type = other RNA
ctgccatggagtatctgaa

SEQ ID NO: 34 - RNA, 21 nt, synthetic construct
  source 1..21: mol_type = other RNA
ttcagatactccatggcagtg

SEQ ID NO: 35 - RNA, 19 nt, synthetic construct
  source 1..19: mol_type = other RNA
ctgccatggagtatctgaa

SEQ ID NO: 36 - RNA, 21 nt, synthetic construct
  source 1..21: mol_type = other RNA
ttcagatactccatggcagtg

SEQ ID NO: 37 - RNA, 19 nt, synthetic construct
  source 1..19: mol_type = other RNA
ctgccatggagtatctgaa

SEQ ID NO: 38 - RNA, 21 nt, synthetic construct
  source 1..21: mol_type = other RNA
ttcagatactccatggcagtg

SEQ ID NO: 39 - RNA, 19 nt, synthetic construct
  source 1..19: mol_type = other RNA
ctgccatggagtatctgaa

SEQ ID NO: 40 - RNA, 21 nt, synthetic construct
  source 1..21: mol_type = other RNA
ttcagatactccatggcagtg

SEQ ID NO: 41 - RNA, 19 nt, synthetic construct
  source 1..19: mol_type = other RNA
ctgccatggagtatctgaa

SEQ ID NO: 42 - RNA, 21 nt, synthetic construct
  source 1..21: mol_type = other RNA
ttcagatactccatggcagtg

SEQ ID NO: 43 - RNA, 19 nt, synthetic construct
  source 1..19: mol_type = other RNA
ctgccatggagtatctgaa

SEQ ID NO: 44 - RNA, 21 nt, synthetic construct
  source 1..21: mol_type = other RNA
ttcagatactccatggcagtg

SEQ ID NO: 45 - RNA, 21 nt, synthetic construct
  source 1..21: mol_type = other RNA
ctgccatggagtatctgaacg

SEQ ID NO: 46 - RNA, 21 nt, synthetic construct
  source 1..21: mol_type = other RNA
ttcagatactccatggcagtg

SEQ ID NO: 47 - RNA, 21 nt, synthetic construct
  source 1..21: mol_type = other RNA
ctgccatggagtatctgaacg

SEQ ID NO: 48 - RNA, 21 nt, synthetic construct
  source 1..21: mol_type = other RNA
ttcagatactccatggcagtg

SEQ ID NO: 49 - RNA, 21 nt, synthetic construct
  source 1..21: mol_type = other RNA
ctgccatggagtatctgaacg

SEQ ID NO: 50 - RNA, 21 nt, synthetic construct
  source 1..21: mol_type = other RNA
ttcagatactccatggcagtg

SEQ ID NO: 51 - RNA, 21 nt, synthetic construct
  source 1..21: mol_type = other RNA
ctgccatggagtatctgaacg

SEQ ID NO: 52 - RNA, 21 nt, synthetic construct
  source 1..21: mol_type = other RNA
ttcagatactccatggcagtg

SEQ ID NO: 53 - RNA, 21 nt, synthetic construct
  source 1..21: mol_type = other RNA
ctgccatggagtatctgaacg

SEQ ID NO: 54 - RNA, 21 nt, synthetic construct
  source 1..21: mol_type = other RNA
ttcagatactccatggcagtg

SEQ ID NO: 55 - RNA, 21 nt, synthetic construct
  source 1..21: mol_type = other RNA
ctgccatggagtatctgaacg

SEQ ID NO: 56 - RNA, 21 nt, synthetic construct
  source 1..21: mol_type = other RNA
ttcagatactccatggcagtg

SEQ ID NO: 57 - RNA, 21 nt, synthetic construct
  source 1..21: mol_type = other RNA
cactgccatggagtatctgaa

SEQ ID NO: 58 - RNA, 23 nt, synthetic construct
  source 1..23: mol_type = other RNA
ttcagatactccatggcagtgac

SEQ ID NO: 59 - RNA, 21 nt, synthetic construct
  source 1..21: mol_type = other RNA
cactgccatggagtatctgaa

SEQ ID NO: 60 - RNA, 23 nt, synthetic construct
  source 1..23: mol_type = other RNA
ttcagatactccatggcagtgac

SEQ ID NO: 61 - RNA, 21 nt, synthetic construct
  source 1..21: mol_type = other RNA
cactgccatggagtatctgaa

SEQ ID NO: 62 - RNA, 23 nt, synthetic construct
  source 1..23: mol_type = other RNA
ttcagatactccatggcagtgac

SEQ ID NO: 63 - RNA, 21 nt, synthetic construct
  source 1..21: mol_type = other RNA
cactgccatggagtatctgaa

SEQ ID NO: 64 - RNA, 23 nt, synthetic construct
  source 1..23: mol_type = other RNA
ttcagatactccatggcagtgac

SEQ ID NO: 65 - RNA, 21 nt, synthetic construct
  source 1..21: mol_type = other RNA
cactgccatggagtatctgaa

SEQ ID NO: 66 - RNA, 23 nt, synthetic construct
  source 1..23: mol_type = other RNA
ttcagatactccatggcagtgac

SEQ ID NO: 67 - RNA, 21 nt, synthetic construct
  source 1..21: mol_type = other RNA
cactgccatggagtatctgaa

SEQ ID NO: 68 - RNA, 23 nt, synthetic construct
  source 1..23: mol_type = other RNA
ttcagatactccatggcagtgac

SEQ ID NO: 69 - RNA, 19 nt, synthetic construct
  source 1..19: mol_type = other RNA
ctgccatggagtatctgaa

SEQ ID NO: 70 - RNA, 21 nt, synthetic construct
  source 1..21: mol_type = other RNA
ttcagatactccatggcagtg

SEQ ID NO: 71 - RNA, 19 nt, synthetic construct
  source 1..19: mol_type = other RNA
ctgccatggagtatctgaa

SEQ ID NO: 72 - RNA, 21 nt, synthetic construct
  source 1..21: mol_type = other RNA
ttcagatactccatggcagtg

SEQ ID NO: 73 - RNA, 19 nt, synthetic construct
  source 1..19: mol_type = other RNA
ctgccatggagtatctgaa

SEQ ID NO: 74 - RNA, 21 nt, synthetic construct
  source 1..21: mol_type = other RNA
ttcagatactccatggcagtg

SEQ ID NO: 75 - RNA, 21 nt, synthetic construct
  source 1..21: mol_type = other RNA
ctgccatggagtatctgaacg

SEQ ID NO: 76 - RNA, 21 nt, synthetic construct
  source 1..21: mol_type = other RNA
ttcagatactccatggcagtg

SEQ ID NO: 77 - RNA, 21 nt, synthetic construct
  source 1..21: mol_type = other RNA
ctgccatggagtatctgaacg

SEQ ID NO: 78 - RNA, 21 nt, synthetic construct
  source 1..21: mol_type = other RNA
ttcagatactccatggcagtg

SEQ ID NO: 79 - RNA, 21 nt, synthetic construct
  source 1..21: mol_type = other RNA
ctgccatggagtatctgaacg

SEQ ID NO: 80 - RNA, 21 nt, synthetic construct
  source 1..21: mol_type = other RNA
ttcagatactccatggcagtg

SEQ ID NO: 81 - RNA, 21 nt, synthetic construct
  source 1..21: mol_type = other RNA
cactgccatggagtatctgaa

SEQ ID NO: 82 - RNA, 23 nt, synthetic construct
  source 1..23: mol_type = other RNA
ttcagatactccatggcagtgac

SEQ ID NO: 83 - RNA, 21 nt, synthetic construct
  source 1..21: mol_type = other RNA
cactgccatggagtatctgaa

SEQ ID NO: 84 - RNA, 23 nt, synthetic construct
  source 1..23: mol_type = other RNA
ttcagatactccatggcagtgac

SEQ ID NO: 85 - RNA, 21 nt, synthetic construct
  source 1..21: mol_type = other RNA
cactgccatggagtatctgaa

SEQ ID NO: 86 - RNA, 23 nt, synthetic construct
  source 1..23: mol_type = other RNA
ttcagatactccatggcagtgac

SEQ ID NO: 87 - RNA, 19 nt, synthetic construct
  source 1..19: mol_type = other RNA
ctgccatggagtatctgaa

SEQ ID NO: 88 - RNA, 21 nt, synthetic construct
  source 1..21: mol_type = other RNA
ttcagatactccatggcagtg

SEQ ID NO: 89 - RNA, 19 nt, synthetic construct
  source 1..19: mol_type = other RNA
ctgccatggagtatctgaa

SEQ ID NO: 90 - RNA, 21 nt, synthetic construct
  source 1..21: mol_type = other RNA
ttcagatactccatggcagtg

SEQ ID NO: 91 - RNA, 19 nt, synthetic construct
  source 1..19: mol_type = other RNA
ctgccatggagtatctgaa

SEQ ID NO: 92 - RNA, 21 nt, synthetic construct
  source 1..21: mol_type = other RNA
ttcagatactccatggcagtg

SEQ ID NO: 93 - RNA, 19 nt, synthetic construct
  source 1..19: mol_type = other RNA
ctgccatggagtatctgaa

SEQ ID NO: 94 - RNA, 21 nt, synthetic construct
  source 1..21: mol_type = other RNA
ttcagatactccatggcagtg

SEQ ID NO: 95 - RNA, 19 nt, synthetic construct
  source 1..19: mol_type = other RNA
ctgccatggagtatctgaa

SEQ ID NO: 96 - RNA, 21 nt, synthetic construct
  source 1..21: mol_type = other RNA
ttcagatactccatggcagtg

SEQ ID NO: 97 - RNA, 19 nt, synthetic construct
  source 1..19: mol_type = other RNA
ctgccatggagtatctgaa

SEQ ID NO: 98 - RNA, 21 nt, synthetic construct
  source 1..21: mol_type = other RNA
ttcagatactccatggcagtg

SEQ ID NO: 99 - RNA, 21 nt, synthetic construct
  source 1..21: mol_type = other RNA
ctgccatggagtatctgaacg

SEQ ID NO: 100 - RNA, 21 nt, synthetic construct
  source 1..21: mol_type = other RNA
ttcagatactccatggcagtg

SEQ ID NO: 101 - RNA, 21 nt, synthetic construct
  source 1..21: mol_type = other RNA
ctgccatggagtatctgaacg

SEQ ID NO: 102 - RNA, 21 nt, synthetic construct
  source 1..21: mol_type = other RNA
ttcagatactccatggcagtg

SEQ ID NO: 103 - RNA, 21 nt, synthetic construct
  source 1..21: mol_type = other RNA
ctgccatggagtatctgaacg

SEQ ID NO: 104 - RNA, 21 nt, synthetic construct
  source 1..21: mol_type = other RNA
ttcagatactccatggcagtg

SEQ ID NO: 105 - RNA, 21 nt, synthetic construct
  source 1..21: mol_type = other RNA
ctgccatggagtatctgaacg

SEQ ID NO: 106 - RNA, 21 nt, synthetic construct
  source 1..21: mol_type = other RNA
ttcagatactccatggcagtg

SEQ ID NO: 107 - RNA, 21 nt, synthetic construct
  source 1..21: mol_type = other RNA
ctgccatggagtatctgaacg

SEQ ID NO: 108 - RNA, 21 nt, synthetic construct
  source 1..21: mol_type = other RNA
ttcagatactccatggcagtg

SEQ ID NO: 109 - RNA, 21 nt, synthetic construct
  source 1..21: mol_type = other RNA
ctgccatggagtatctgaacg

SEQ ID NO: 110 - RNA, 21 nt, synthetic construct
  source 1..21: mol_type = other RNA
ttcagatactccatggcagtg

SEQ ID NO: 111 - RNA, 21 nt, synthetic construct
  source 1..21: mol_type = other RNA
cactgccatggagtatctgaa

SEQ ID NO: 112 - RNA, 23 nt, synthetic construct
  source 1..23: mol_type = other RNA
ttcagatactccatggcagtgac

SEQ ID NO: 113 - RNA, 21 nt, synthetic construct
  source 1..21: mol_type = other RNA
cactgccatggagtatctgaa

SEQ ID NO: 114 - RNA, 23 nt, synthetic construct
  source 1..23: mol_type = other RNA
ttcagatactccatggcagtgac

SEQ ID NO: 115 - RNA, 21 nt, synthetic construct
  source 1..21: mol_type = other RNA
cactgccatggagtatctgaa

SEQ ID NO: 116 - RNA, 23 nt, synthetic construct
  source 1..23: mol_type = other RNA
ttcagatactccatggcagtgac

SEQ ID NO: 117 - RNA, 21 nt, synthetic construct
  source 1..21: mol_type = other RNA
cactgccatggagtatctgaa

SEQ ID NO: 118 - RNA, 23 nt, synthetic construct
  source 1..23: mol_type = other RNA
ttcagatactccatggcagtgac

SEQ ID NO: 119 - RNA, 21 nt, synthetic construct
  source 1..21: mol_type = other RNA
cactgccatggagtatctgaa

SEQ ID NO: 120 - RNA, 23 nt, synthetic construct
  source 1..23: mol_type = other RNA
ttcagatactccatggcagtgac

SEQ ID NO: 121 - RNA, 21 nt, synthetic construct
  source 1..21: mol_type = other RNA
cactgccatggagtatctgaa

SEQ ID NO: 122 - RNA, 23 nt, synthetic construct
  source 1..23: mol_type = other RNA
ttcagatactccatggcagtgac

SEQ ID NO: 123 - RNA, 19 nt, synthetic construct
  source 1..19: mol_type = other RNA
acaacatcaagtactacga

SEQ ID NO: 124 - RNA, 19 nt, synthetic construct
  source 1..19: mol_type = other RNA
tcgtagtacttgatgttgt

SEQ ID NO: 125 - RNA, 19 nt, synthetic construct
  source 1..19: mol_type = other RNA
acaacatcaagtactacgn

SEQ ID NO: 126 - RNA, 19 nt, synthetic construct
  source 1..19: mol_type = other RNA
ncgtagtacttgatgttgt

SEQ ID NO: 127 - RNA, 19 nt, synthetic construct
  source 1..19: mol_type = other RNA
acaacatcaagtactacgn

SEQ ID NO: 128 - RNA, 21 nt, synthetic construct
  source 1..21: mol_type = other RNA
ncgtagtacttgatgttgttg

SEQ ID NO: 129 - RNA, 21 nt, synthetic construct
  source 1..21: mol_type = other RNA
caacaacatcaagtactacgn

SEQ ID NO: 130 - RNA, 23 nt, synthetic construct
  source 1..23: mol_type = other RNA
ncgtagtacttgatgttgttgat

SEQ ID NO: 131 - RNA, 19 nt, synthetic construct
  source 1..19: mol_type = other RNA
acaacatcaagtactacga

SEQ ID NO: 132 - RNA, 21 nt, synthetic construct
  source 1..21: mol_type = other RNA
tcgtagtacttgatgttgttg

SEQ ID NO: 133 - RNA, 21 nt, synthetic construct
  source 1..21: mol_type = other RNA
acaacatcaagtactacgacg

SEQ ID NO: 134 - RNA, 21 nt, synthetic construct
  source 1..21: mol_type = other RNA
tcgtagtacttgatgttgttg

SEQ ID NO: 135 - RNA, 21 nt, synthetic construct
  source 1..21: mol_type = other RNA
gtacaacatcaagtactacga

SEQ ID NO: 136 - RNA, 23 nt, synthetic construct
  source 1..23: mol_type = other RNA
tcgtagtacttgatgttgttgat

SEQ ID NO: 137 - RNA, 19 nt, synthetic construct
  source 1..19: mol_type = other RNA
acaacatcaagtactacga

SEQ ID NO: 138 - RNA, 21 nt, synthetic construct
  source 1..21: mol_type = other RNA
tcgtagtacttgatgttgttg

SEQ ID NO: 139 - RNA, 19 nt, synthetic construct
  source 1..19: mol_type = other RNA
acaacatcaagtactacga

SEQ ID NO: 140 - RNA, 21 nt, synthetic construct
  source 1..21: mol_type = other RNA
tcgtagtacttgatgttgttg

SEQ ID NO: 141 - RNA, 19 nt, synthetic construct
  source 1..19: mol_type = other RNA
acaacatcaagtactacga

SEQ ID NO: 142 - RNA, 21 nt, synthetic construct
  source 1..21: mol_type = other RNA
tcgtagtacttgatgttgttg

SEQ ID NO: 143 - RNA, 21 nt, synthetic construct
  source 1..21: mol_type = other RNA
acaacatcaagtactacgacg

SEQ ID NO: 144 - RNA, 21 nt, synthetic construct
  source 1..21: mol_type = other RNA
tcgtagtacttgatgttgttg

SEQ ID NO: 145 - RNA, 21 nt, synthetic construct
  source 1..21: mol_type = other RNA
acaacatcaagtactacgacg

SEQ ID NO: 146 - RNA, 21 nt, synthetic construct
  source 1..21: mol_type = other RNA
tcgtagtacttgatgttgttg

SEQ ID NO: 147 - RNA, 21 nt, synthetic construct
  source 1..21: mol_type = other RNA
acaacatcaagtactacgacg

SEQ ID NO: 148 - RNA, 21 nt, synthetic construct
  source 1..21: mol_type = other RNA
tcgtagtacttgatgttgttg

SEQ ID NO: 149 - RNA, 21 nt, synthetic construct
  source 1..21: mol_type = other RNA
gtacaacatcaagtactacga

SEQ ID NO: 150 - RNA, 23 nt, synthetic construct
  source 1..23: mol_type = other RNA
tcgtagtacttgatgttgttgat

SEQ ID NO: 151 - RNA, 21 nt, synthetic construct
  source 1..21: mol_type = other RNA
gtacaacatcaagtactacga

SEQ ID NO: 152 - RNA, 23 nt, synthetic construct
  source 1..23: mol_type = other RNA
tcgtagtacttgatgttgttgat

SEQ ID NO: 153 - RNA, 21 nt, synthetic construct
  source 1..21: mol_type = other RNA
gtacaacatcaagtactacga

SEQ ID NO: 154 - RNA, 23 nt, synthetic construct
  source 1..23: mol_type = other RNA
tcgtagtacttgatgttgttgat

SEQ ID NO: 155 - RNA, 19 nt, synthetic construct
  source 1..19: mol_type = other RNA
acaacatcaagtactacga

SEQ ID NO: 156 - RNA, 21 nt, synthetic construct
  source 1..21: mol_type = other RNA
tcgtagtacttgatgttgttg

SEQ ID NO: 157 - RNA, 19 nt, synthetic construct
  source 1..19: mol_type = other RNA
acaacatcaagtactacga

SEQ ID NO: 158 - RNA, 21 nt, synthetic construct
  source 1..21: mol_type = other RNA
tcgtagtacttgatgttgttg

SEQ ID NO: 159 - RNA, 19 nt, synthetic construct
  source 1..19: mol_type = other RNA
acaacatcaagtactacga

SEQ ID NO: 160 - RNA, 21 nt, synthetic construct
  source 1..21: mol_type = other RNA
tcgtagtacttgatgttgttg

SEQ ID NO: 161 - RNA, 19 nt, synthetic construct
  source 1..19: mol_type = other RNA
acaacatcaagtactacga

SEQ ID NO: 162 - RNA, 21 nt, synthetic construct
  source 1..21: mol_type = other RNA
tcgtagtacttgatgttgttg

SEQ ID NO: 163 - RNA, 19 nt, synthetic construct
  source 1..19: mol_type = other RNA
acaacatcaagtactacga

SEQ ID NO: 164 - RNA, 21 nt, synthetic construct
  source 1..21: mol_type = other RNA
tcgtagtacttgatgttgttg

SEQ ID NO: 165 - RNA, 19 nt, synthetic construct
  source 1..19: mol_type = other RNA
acaacatcaagtactacga

SEQ ID NO: 166 - RNA, 21 nt, synthetic construct
  source 1..21: mol_type = other RNA
tcgtagtacttgatgttgttg

SEQ ID NO: 167 - RNA, 21 nt, synthetic construct
  source 1..21: mol_type = other RNA
acaacatcaagtactacgacg

SEQ ID NO: 168 - RNA, 21 nt, synthetic construct
  source 1..21: mol_type = other RNA
tcgtagtacttgatgttgttg

SEQ ID NO: 169 - RNA, 21 nt, synthetic construct
  source 1..21: mol_type = other RNA
acaacatcaagtactacgacg

SEQ ID NO: 170 - RNA, 21 nt, synthetic construct
  source 1..21: mol_type = other RNA
tcgtagtacttgatgttgttg

SEQ ID NO: 171 - RNA, 21 nt, synthetic construct
  source 1..21: mol_type = other RNA
acaacatcaagtactacgacg

SEQ ID NO: 172 - RNA, 21 nt, synthetic construct
  source 1..21: mol_type = other RNA
tcgtagtacttgatgttgttg

SEQ ID NO: 173 - RNA, 21 nt, synthetic construct
  source 1..21: mol_type = other RNA
acaacatcaagtactacgacg

SEQ ID NO: 174 - RNA, 21 nt, synthetic construct
  source 1..21: mol_type = other RNA
tcgtagtacttgatgttgttg

SEQ ID NO: 175 - RNA, 21 nt, synthetic construct
  source 1..21: mol_type = other RNA
acaacatcaagtactacgacg

SEQ ID NO: 176 - RNA, 21 nt, synthetic construct
  source 1..21: mol_type = other RNA
tcgtagtacttgatgttgttg

SEQ ID NO: 177 - RNA, 21 nt, synthetic construct
  source 1..21: mol_type = other RNA
acaacatcaagtactacgacg

SEQ ID NO: 178 - RNA, 21 nt, synthetic construct
  source 1..21: mol_type = other RNA
tcgtagtacttgatgttgttg

SEQ ID NO: 179 - RNA, 21 nt, synthetic construct
  source 1..21: mol_type = other RNA
gtacaacatcaagtactacga

SEQ ID NO: 180 - RNA, 23 nt, synthetic construct
  source 1..23: mol_type = other RNA
tcgtagtacttgatgttgttgat

SEQ ID NO: 181 - RNA, 21 nt, synthetic construct
  source 1..21: mol_type = other RNA
gtacaacatcaagtactacga

SEQ ID NO: 182 - RNA, 23 nt, synthetic construct
  source 1..23: mol_type = other RNA
tcgtagtacttgatgttgttgat

SEQ ID NO: 183 - RNA, 21 nt, synthetic construct
  source 1..21: mol_type = other RNA
gtacaacatcaagtactacga

SEQ ID NO: 184 - RNA, 23 nt, synthetic construct
  source 1..23: mol_type = other RNA
tcgtagtacttgatgttgttgat

SEQ ID NO: 185 - RNA, 21 nt, synthetic construct
  source 1..21: mol_type = other RNA
gtacaacatcaagtactacga

SEQ ID NO: 186 - RNA, 23 nt, synthetic construct
  source 1..23: mol_type = other RNA
tcgtagtacttgatgttgttgat

SEQ ID NO: 187 - RNA, 21 nt, synthetic construct
  source 1..21: mol_type = other RNA
gtacaacatcaagtactacga

SEQ ID NO: 188 - RNA, 23 nt, synthetic construct
  source 1..23: mol_type = other RNA
tcgtagtacttgatgttgttgat

SEQ ID NO: 189 - RNA, 21 nt, synthetic construct
  source 1..21: mol_type = other RNA
gtacaacatcaagtactacga

SEQ ID NO: 190 - RNA, 23 nt, synthetic construct
  source 1..23: mol_type = other RNA
tcgtagtacttgatgttgttgat

SEQ ID NO: 191 - RNA, 19 nt, synthetic construct
  source 1..19: mol_type = other RNA
acaacatcaagtactacga

SEQ ID NO: 192 - RNA, 21 nt, synthetic construct
  source 1..21: mol_type = other RNA
tcgtagtacttgatgttgttg

SEQ ID NO: 193 - RNA, 19 nt, synthetic construct
  source 1..19: mol_type = other RNA
acaacatcaagtactacga

SEQ ID NO: 194 - RNA, 21 nt, synthetic construct
  source 1..21: mol_type = other RNA
tcgtagtacttgatgttgttg

SEQ ID NO: 195 - RNA, 19 nt, synthetic construct
  source 1..19: mol_type = other RNA
acaacatcaagtactacga

SEQ ID NO: 196 - RNA, 21 nt, synthetic construct
  source 1..21: mol_type = other RNA
tcgtagtacttgatgttgttg

SEQ ID NO: 197 - RNA, 21 nt, synthetic construct
  source 1..21: mol_type = other RNA
acaacatcaagtactacgacg

SEQ ID NO: 198 - RNA, 21 nt, synthetic construct
  source 1..21: mol_type = other RNA
tcgtagtacttgatgttgttg

SEQ ID NO: 199 - RNA, 21 nt, synthetic construct
  source 1..21: mol_type = other RNA
acaacatcaagtactacgacg

SEQ ID NO: 200 - RNA, 21 nt, synthetic construct
  source 1..21: mol_type = other RNA
tcgtagtacttgatgttgttg

SEQ ID NO: 201 - RNA, 21 nt, synthetic construct
  source 1..21: mol_type = other RNA
acaacatcaagtactacgacg

SEQ ID NO: 202 - RNA, 21 nt, synthetic construct
  source 1..21: mol_type = other RNA
tcgtagtacttgatgttgttg

SEQ ID NO: 203 - RNA, 21 nt, synthetic construct
  source 1..21: mol_type = other RNA
gtacaacatcaagtactacga

SEQ ID NO: 204 - RNA, 23 nt, synthetic construct
  source 1..23: mol_type = other RNA
tcgtagtacttgatgttgttgat

SEQ ID NO: 205 - RNA, 21 nt, synthetic construct
  source 1..21: mol_type = other RNA
gtacaacatcaagtactacga

SEQ ID NO: 206 - RNA, 23 nt, synthetic construct
  source 1..23: mol_type = other RNA
tcgtagtacttgatgttgttgat

SEQ ID NO: 207 - RNA, 21 nt, synthetic construct
  source 1..21: mol_type = other RNA
gtacaacatcaagtactacga

SEQ ID NO: 208 - RNA, 23 nt, synthetic construct
  source 1..23: mol_type = other RNA
tcgtagtacttgatgttgttgat

SEQ ID NO: 209 - RNA, 19 nt, synthetic construct
  source 1..19: mol_type = other RNA
acaacatcaagtactacga

SEQ ID NO: 210 - RNA, 21 nt, synthetic construct
  source 1..21: mol_type = other RNA
tcgtagtacttgatgttgttg

SEQ ID NO: 211 - RNA, 19 nt, synthetic construct
  source 1..19: mol_type = other RNA
acaacatcaagtactacga

SEQ ID NO: 212 - RNA, 21 nt, synthetic construct
  source 1..21: mol_type = other RNA
tcgtagtacttgatgttgttg

SEQ ID NO: 213 - RNA, 19 nt, synthetic construct
  source 1..19: mol_type = other RNA
acaacatcaagtactacga

SEQ ID NO: 214 - RNA, 21 nt, synthetic construct
  source 1..21: mol_type = other RNA
tcgtagtacttgatgttgttg

SEQ ID NO: 215 - RNA, 19 nt, synthetic construct
  source 1..19: mol_type = other RNA
acaacatcaagtactacga

SEQ ID NO: 216 - RNA, 21 nt, synthetic construct
  source 1..21: mol_type = other RNA
tcgtagtacttgatgttgttg

SEQ ID NO: 217 - RNA, 19 nt, synthetic construct
  source 1..19: mol_type = other RNA
acaacatcaagtactacga

SEQ ID NO: 218 - RNA, 21 nt, synthetic construct
  source 1..21: mol_type = other RNA
tcgtagtacttgatgttgttg

SEQ ID NO: 219 - RNA, 19 nt, synthetic construct
  source 1..19: mol_type = other RNA
acaacatcaagtactacga

SEQ ID NO: 220 - RNA, 21 nt, synthetic construct
  source 1..21: mol_type = other RNA
tcgtagtacttgatgttgttg

SEQ ID NO: 221 - RNA, 21 nt, synthetic construct
  source 1..21: mol_type = other RNA
acaacatcaagtactacgacg

SEQ ID NO: 222 - RNA, 21 nt, synthetic construct
  source 1..21: mol_type = other RNA
tcgtagtacttgatgttgttg

SEQ ID NO: 223 - RNA, 21 nt, synthetic construct
  source 1..21: mol_type = other RNA
acaacatcaagtactacgacg

SEQ ID NO: 224 - RNA, 21 nt, synthetic construct
  source 1..21: mol_type = other RNA
tcgtagtacttgatgttgttg

SEQ ID NO: 225 - RNA, 21 nt, synthetic construct
  source 1..21: mol_type = other RNA
acaacatcaagtactacgacg

SEQ ID NO: 226 - RNA, 21 nt, synthetic construct
  source 1..21: mol_type = other RNA
tcgtagtacttgatgttgttg

SEQ ID NO: 227 - RNA, 21 nt, synthetic construct
  source 1..21: mol_type = other RNA
acaacatcaagtactacgacg

SEQ ID NO: 228 - RNA, 21 nt, synthetic construct
  source 1..21: mol_type = other RNA
tcgtagtacttgatgttgttg

SEQ ID NO: 229 - RNA, 21 nt, synthetic construct
  source 1..21: mol_type = other RNA
acaacatcaagtactacgacg

SEQ ID NO: 230 - RNA, 21 nt, synthetic construct
  source 1..21: mol_type = other RNA
tcgtagtacttgatgttgttg

SEQ ID NO: 231 - RNA, 21 nt, synthetic construct
  source 1..21: mol_type = other RNA
acaacatcaagtactacgacg

SEQ ID NO: 232 - RNA, 21 nt, synthetic construct
  source 1..21: mol_type = other RNA
tcgtagtacttgatgttgttg

SEQ ID NO: 233 - RNA, 21 nt, synthetic construct
  source 1..21: mol_type = other RNA
gtacaacatcaagtactacga

SEQ ID NO: 234 - RNA, 23 nt, synthetic construct
  source 1..23: mol_type = other RNA
tcgtagtacttgatgttgttgat

SEQ ID NO: 235 - RNA, 21 nt, synthetic construct
  source 1..21: mol_type = other RNA
gtacaacatcaagtactacga

SEQ ID NO: 236 - RNA, 23 nt, synthetic construct
  source 1..23: mol_type = other RNA
tcgtagtacttgatgttgttgat

SEQ ID NO: 237 - RNA, 21 nt, synthetic construct
  source 1..21: mol_type = other RNA
gtacaacatcaagtactacga

SEQ ID NO: 238 - RNA, 23 nt, synthetic construct
  source 1..23: mol_type = other RNA
tcgtagtacttgatgttgttgat

SEQ ID NO: 239 - RNA, 21 nt, synthetic construct
  source 1..21: mol_type = other RNA
gtacaacatcaagtactacga

SEQ ID NO: 240 - RNA, 23 nt, synthetic construct
  source 1..23: mol_type = other RNA
tcgtagtacttgatgttgttgat

SEQ ID NO: 241 - RNA, 21 nt, synthetic construct
  source 1..21: mol_type = other RNA
gtacaacatcaagtactacga

SEQ ID NO: 242 - RNA, 23 nt, synthetic construct
  source 1..23: mol_type = other RNA
tcgtagtacttgatgttgttgat

SEQ ID NO: 243 - RNA, 21 nt, synthetic construct
  source 1..21: mol_type = other RNA
gtacaacatcaagtactacga

SEQ ID NO: 244 - RNA, 23 nt, synthetic construct
  source 1..23: mol_type = other RNA
tcgtagtacttgatgttgttgat

SEQ ID NO: 245 - RNA, 19 nt, synthetic construct
  source 1..19: mol_type = other RNA
cgactactacatctccgtg

SEQ ID NO: 246 - RNA, 19 nt, synthetic construct
  source 1..19: mol_type = other RNA
cacggagatgtagtagtcg

SEQ ID NO: 247 - RNA, 19 nt, synthetic construct
  source 1..19: mol_type = other RNA
cgactactacatctccgtn

SEQ ID NO: 248 - RNA, 19 nt, synthetic construct
  source 1..19: mol_type = other RNA
nacggagatgtagtagtcg

SEQ ID NO: 249 - RNA, 19 nt, synthetic construct
  source 1..19: mol_type = other RNA
cgactactacatctccgtn

SEQ ID NO: 250 - RNA, 21 nt, synthetic construct
  source 1..21: mol_type = other RNA
nacggagatgtagtagtcgtt

SEQ ID NO: 251 - RNA, 21 nt, synthetic construct
  source 1..21: mol_type = other RNA
aacgactactacatctccgtn

SEQ ID NO: 252 - RNA, 23 nt, synthetic construct
  source 1..23: mol_type = other RNA
nacggagatgtagtagtcgttgc

SEQ ID NO: 253 - RNA, 19 nt, synthetic construct
  source 1..19: mol_type = other RNA
cgactactacatctccgtg

SEQ ID NO: 254 - RNA, 21 nt, synthetic construct
  source 1..21: mol_type = other RNA
cacggagatgtagtagtcgtt

SEQ ID NO: 255 - RNA, 21 nt, synthetic construct
  source 1..21: mol_type = other RNA
cgactactacatctccgtgta

SEQ ID NO: 256 - RNA, 21 nt, synthetic construct
  source 1..21: mol_type = other RNA
cacggagatgtagtagtcgtt

SEQ ID NO: 257 - RNA, 21 nt, synthetic construct
  source 1..21: mol_type = other RNA
cgcgactactacatctccgtg

SEQ ID NO: 258 - RNA, 23 nt, synthetic construct
  source 1..23: mol_type = other RNA
cacggagatgtagtagtcgttgc

SEQ ID NO: 259 - RNA, 19 nt, synthetic construct
  source 1..19: mol_type = other RNA
cgactactacatctccgtg

SEQ ID NO: 260 - RNA, 21 nt, synthetic construct
  source 1..21: mol_type = other RNA
cacggagatgtagtagtcgtt

SEQ ID NO: 261 - RNA, 19 nt, synthetic construct
  source 1..19: mol_type = other RNA
cgactactacatctccgtg

SEQ ID NO: 262 - RNA, 21 nt, synthetic construct
  source 1..21: mol_type = other RNA
cacggagatgtagtagtcgtt

SEQ ID NO: 263 - RNA, 19 nt, synthetic construct
  source 1..19: mol_type = other RNA
cgactactacatctccgtg

SEQ ID NO: 264 - RNA, 21 nt, synthetic construct
  source 1..21: mol_type = other RNA
cacggagatgtagtagtcgtt

SEQ ID NO: 265 - RNA, 21 nt, synthetic construct
  source 1..21: mol_type = other RNA
cgactactacatctccgtgta

SEQ ID NO: 266 - RNA, 21 nt, synthetic construct
  source 1..21: mol_type = other RNA
cacggagatgtagtagtcgtt

SEQ ID NO: 267 - RNA, 21 nt, synthetic construct
  source 1..21: mol_type = other RNA
cgactactacatctccgtgta

SEQ ID NO: 268 - RNA, 21 nt, synthetic construct
  source 1..21: mol_type = other RNA
cacggagatgtagtagtcgtt

SEQ ID NO: 269 - RNA, 21 nt, synthetic construct
  source 1..21: mol_type = other RNA
cgactactacatctccgtgta

SEQ ID NO: 270 - RNA, 21 nt, synthetic construct
  source 1..21: mol_type = other RNA
cacggagatgtagtagtcgtt

SEQ ID NO: 271 - RNA, 21 nt, synthetic construct
  source 1..21: mol_type = other RNA
cgcgactactacatctccgtg

SEQ ID NO: 272 - RNA, 23 nt, synthetic construct
  source 1..23: mol_type = other RNA
cacggagatgtagtagtcgttgc

SEQ ID NO: 273 - RNA, 21 nt, synthetic construct
  source 1..21: mol_type = other RNA
cgcgactactacatctccgtg

SEQ ID NO: 274 - RNA, 23 nt, synthetic construct
  source 1..23: mol_type = other RNA
cacggagatgtagtagtcgttgc

SEQ ID NO: 275 - RNA, 21 nt, synthetic construct
  source 1..21: mol_type = other RNA
cgcgactactacatctccgtg

SEQ ID NO: 276 - RNA, 23 nt, synthetic construct
  source 1..23: mol_type = other RNA
cacggagatgtagtagtcgttgc

SEQ ID NO: 277 - RNA, 19 nt, synthetic construct
  source 1..19: mol_type = other RNA
cgactactacatctccgtg

SEQ ID NO: 278 - RNA, 21 nt, synthetic construct
  source 1..21: mol_type = other RNA
cacggagatgtagtagtcgtt

SEQ ID NO: 279 - RNA, 19 nt, synthetic construct
  source 1..19: mol_type = other RNA
cgactactacatctccgtg

SEQ ID NO: 280 - RNA, 21 nt, synthetic construct
  source 1..21: mol_type = other RNA
cacggagatgtagtagtcgtt

SEQ ID NO: 281 - RNA, 19 nt, synthetic construct
  source 1..19: mol_type = other RNA
cgactactacatctccgtg

SEQ ID NO: 282 - RNA, 21 nt, synthetic construct
  source 1..21: mol_type = other RNA
cacggagatgtagtagtcgtt

SEQ ID NO: 283 - RNA, 19 nt, synthetic construct
  source 1..19: mol_type = other RNA
cgactactacatctccgtg

SEQ ID NO: 284 - RNA, 21 nt, synthetic construct
  source 1..21: mol_type = other RNA
cacggagatgtagtagtcgtt

SEQ ID NO: 285 - RNA, 19 nt, synthetic construct
  source 1..19: mol_type = other RNA
cgactactacatctccgtg

SEQ ID NO: 286 - RNA, 21 nt, synthetic construct
  source 1..21: mol_type = other RNA
cacggagatgtagtagtcgtt

SEQ ID NO: 287 - RNA, 19 nt, synthetic construct
  source 1..19: mol_type = other RNA
cgactactacatctccgtg

SEQ ID NO: 288 - RNA, 21 nt, synthetic construct
  source 1..21: mol_type = other RNA
cacggagatgtagtagtcgtt

SEQ ID NO: 289 - RNA, 21 nt, synthetic construct
  source 1..21: mol_type = other RNA
cgactactacatctccgtgta

SEQ ID NO: 290 - RNA, 21 nt, synthetic construct
  source 1..21: mol_type = other RNA
cacggagatgtagtagtcgtt

SEQ ID NO: 291 - RNA, 21 nt, synthetic construct
  source 1..21: mol_type = other RNA
cgactactacatctccgtgta

SEQ ID NO: 292 - RNA, 21 nt, synthetic construct
  source 1..21: mol_type = other RNA
cacggagatgtagtagtcgtt

SEQ ID NO: 293 - RNA, 21 nt, synthetic construct
  source 1..21: mol_type = other RNA
cgactactacatctccgtgta

SEQ ID NO: 294 - RNA, 21 nt, synthetic construct
  source 1..21: mol_type = other RNA
cacggagatgtagtagtcgtt

SEQ ID NO: 295 - RNA, 21 nt, synthetic construct
  source 1..21: mol_type = other RNA
cgactactacatctccgtgta

SEQ ID NO: 296 - RNA, 21 nt, synthetic construct
  source 1..21: mol_type = other RNA
cacggagatgtagtagtcgtt

SEQ ID NO: 297 - RNA, 21 nt, synthetic construct
  source 1..21: mol_type = other RNA
cgactactacatctccgtgta

SEQ ID NO: 298 - RNA, 21 nt, synthetic construct
  source 1..21: mol_type = other RNA
cacggagatgtagtagtcgtt

SEQ ID NO: 299 - RNA, 21 nt, synthetic construct
  source 1..21: mol_type = other RNA
cgactactacatctccgtgta

SEQ ID NO: 300 - RNA, 21 nt, synthetic construct
  source 1..21: mol_type = other RNA
cacggagatgtagtagtcgtt

SEQ ID NO: 301 - RNA, 21 nt, synthetic construct
  source 1..21: mol_type = other RNA
cgcgactactacatctccgtg

SEQ ID NO: 302 - RNA, 23 nt, synthetic construct
  source 1..23: mol_type = other RNA
cacggagatgtagtagtcgttgc

SEQ ID NO: 303 - RNA, 21 nt, synthetic construct
  source 1..21: mol_type = other RNA
cgcgactactacatctccgtg

SEQ ID NO: 304 - RNA, 23 nt, synthetic construct
  source 1..23: mol_type = other RNA
cacggagatgtagtagtcgttgc

SEQ ID NO: 305 - RNA, 21 nt, synthetic construct
  source 1..21: mol_type = other RNA
cgcgactactacatctccgtg

SEQ ID NO: 306 - RNA, 23 nt, synthetic construct
  source 1..23: mol_type = other RNA
cacggagatgtagtagtcgttgc

SEQ ID NO: 307 - RNA, 21 nt, synthetic construct
  source 1..21: mol_type = other RNA
cgcgactactacatctccgtg

SEQ ID NO: 308 - RNA, 23 nt, synthetic construct
  source 1..23: mol_type = other RNA
cacggagatgtagtagtcgttgc

SEQ ID NO: 309 - RNA, 21 nt, synthetic construct
  source 1..21: mol_type = other RNA
cgcgactactacatctccgtg

SEQ ID NO: 310 - RNA, 23 nt, synthetic construct
  source 1..23: mol_type = other RNA
cacggagatgtagtagtcgttgc

SEQ ID NO: 311 - RNA, 21 nt, synthetic construct
  source 1..21: mol_type = other RNA
cgcgactactacatctccgtg

SEQ ID NO: 312 - RNA, 23 nt, synthetic construct
  source 1..23: mol_type = other RNA
cacggagatgtagtagtcgttgc

SEQ ID NO: 313 - RNA, 19 nt, synthetic construct
  source 1..19: mol_type = other RNA
cgactactacatctccgtg

SEQ ID NO: 314 - RNA, 21 nt, synthetic construct
  source 1..21: mol_type = other RNA
cacggagatgtagtagtcgtt

SEQ ID NO: 315 - RNA, 19 nt, synthetic construct
  source 1..19: mol_type = other RNA
cgactactacatctccgtg

SEQ ID NO: 316 - RNA, 21 nt, synthetic construct
  source 1..21: mol_type = other RNA
cacggagatgtagtagtcgtt

SEQ ID NO: 317 - RNA, 19 nt, synthetic construct
  source 1..19: mol_type = other RNA
cgactactacatctccgtg

SEQ ID NO: 318 - RNA, 21 nt, synthetic construct
  source 1..21: mol_type = other RNA
cacggagatgtagtagtcgtt

SEQ ID NO: 319 - RNA, 21 nt, synthetic construct
  source 1..21: mol_type = other RNA
cgactactacatctccgtgta

SEQ ID NO: 320 - RNA, 21 nt, synthetic construct
  source 1..21: mol_type = other RNA
cacggagatgtagtagtcgtt

SEQ ID NO: 321 - RNA, 21 nt, synthetic construct
  source 1..21: mol_type = other RNA
cgactactacatctccgtgta

SEQ ID NO: 322 - RNA, 21 nt, synthetic construct
  source 1..21: mol_type = other RNA
cacggagatgtagtagtcgtt

SEQ ID NO: 323 - RNA, 21 nt, synthetic construct
  source 1..21: mol_type = other RNA
cgactactacatctccgtgta

SEQ ID NO: 324 - RNA, 21 nt, synthetic construct
  source 1..21: mol_type = other RNA
cacggagatgtagtagtcgtt

SEQ ID NO: 325 - RNA, 21 nt, synthetic construct
  source 1..21: mol_type = other RNA
cgcgactactacatctccgtg

SEQ ID NO: 326 - RNA, 23 nt, synthetic construct
  source 1..23: mol_type = other RNA
cacggagatgtagtagtcgttgc

SEQ ID NO: 327 - RNA, 21 nt, synthetic construct
  source 1..21: mol_type = other RNA
cgcgactactacatctccgtg

SEQ ID NO: 328 - RNA, 23 nt, synthetic construct
  source 1..23: mol_type = other RNA
cacggagatgtagtagtcgttgc

SEQ ID NO: 329 - RNA, 21 nt, synthetic construct
  source 1..21: mol_type = other RNA
cgcgactactacatctccgtg

SEQ ID NO: 330 - RNA, 23 nt, synthetic construct
  source 1..23: mol_type = other RNA
cacggagatgtagtagtcgttgc

SEQ ID NO: 331 - RNA, 19 nt, synthetic construct
  source 1..19: mol_type = other RNA
cgactactacatctccgtg

SEQ ID NO: 332 - RNA, 21 nt, synthetic construct
  source 1..21: mol_type = other RNA
cacggagatgtagtagtcgtt

SEQ ID NO: 333 - RNA, 19 nt, synthetic construct
  source 1..19: mol_type = other RNA
cgactactacatctccgtg

SEQ ID NO: 334 - RNA, 21 nt, synthetic construct
  source 1..21: mol_type = other RNA
cacggagatgtagtagtcgtt

SEQ ID NO: 335 - RNA, 19 nt, synthetic construct
  source 1..19: mol_type = other RNA
cgactactacatctccgtg

SEQ ID NO: 336 - RNA, 21 nt, synthetic construct
  source 1..21: mol_type = other RNA
cacggagatgtagtagtcgtt

SEQ ID NO: 337 - RNA, 19 nt, synthetic construct
  source 1..19: mol_type = other RNA
cgactactacatctccgtg

SEQ ID NO: 338 - RNA, 21 nt, synthetic construct
  source 1..21: mol_type = other RNA
cacggagatgtagtagtcgtt

SEQ ID NO: 339 - RNA, 19 nt, synthetic construct
  source 1..19: mol_type = other RNA
cgactactacatctccgtg

SEQ ID NO: 340 - RNA, 21 nt, synthetic construct
  source 1..21: mol_type = other RNA
cacggagatgtagtagtcgtt

SEQ ID NO: 341 - RNA, 19 nt, synthetic construct
  source 1..19: mol_type = other RNA
cgactactacatctccgtg

SEQ ID NO: 342 - RNA, 21 nt, synthetic construct
  source 1..21: mol_type = other RNA
cacggagatgtagtagtcgtt

SEQ ID NO: 343 - RNA, 21 nt, synthetic construct
  source 1..21: mol_type = other RNA
cgactactacatctccgtgta

SEQ ID NO: 344 - RNA, 21 nt, synthetic construct
  source 1..21: mol_type = other RNA
cacggagatgtagtagtcgtt

SEQ ID NO: 345 - RNA, 21 nt, synthetic construct
  source 1..21: mol_type = other RNA
cgactactacatctccgtgta

SEQ ID NO: 346 - RNA, 21 nt, synthetic construct
  source 1..21: mol_type = other RNA
cacggagatgtagtagtcgtt

SEQ ID NO: 347 - RNA, 21 nt, synthetic construct
  source 1..21: mol_type = other RNA
cgactactacatctccgtgta

SEQ ID NO: 348 - RNA, 21 nt, synthetic construct
  source 1..21: mol_type = other RNA
cacggagatgtagtagtcgtt

SEQ ID NO: 349 - RNA, 21 nt, synthetic construct
  source 1..21: mol_type = other RNA
cgactactacatctccgtgta

SEQ ID NO: 350 - RNA, 21 nt, synthetic construct
  source 1..21: mol_type = other RNA
cacggagatgtagtagtcgtt

SEQ ID NO: 351 - RNA, 21 nt, synthetic construct
  source 1..21: mol_type = other RNA
cgactactacatctccgtgta

SEQ ID NO: 352 - RNA, 21 nt, synthetic construct
  source 1..21: mol_type = other RNA
cacggagatgtagtagtcgtt

SEQ ID NO: 353 - RNA, 21 nt, synthetic construct
  source 1..21: mol_type = other RNA
cgactactacatctccgtgta

SEQ ID NO: 354 - RNA, 21 nt, synthetic construct
  source 1..21: mol_type = other RNA
cacggagatgtagtagtcgtt

SEQ ID NO: 355 - RNA, 21 nt, synthetic construct
  source 1..21: mol_type = other RNA
cgcgactactacatctccgtg

SEQ ID NO: 356 - RNA, 23 nt, synthetic construct
  source 1..23: mol_type = other RNA
cacggagatgtagtagtcgttgc

SEQ ID NO: 357 - RNA, 21 nt, synthetic construct
  source 1..21: mol_type = other RNA
cgcgactactacatctccgtg

SEQ ID NO: 358 - RNA, 23 nt, synthetic construct
  source 1..23: mol_type = other RNA
cacggagatgtagtagtcgttgc

SEQ ID NO: 359 - RNA, 21 nt, synthetic construct
  source 1..21: mol_type = other RNA
cgcgactactacatctccgtg

SEQ ID NO: 360 - RNA, 23 nt, synthetic construct
  source 1..23: mol_type = other RNA
cacggagatgtagtagtcgttgc

SEQ ID NO: 361 - RNA, 21 nt, synthetic construct
  source 1..21: mol_type = other RNA
cgcgactactacatctccgtg

SEQ ID NO: 362 - RNA, 23 nt, synthetic construct
  source 1..23: mol_type = other RNA
cacggagatgtagtagtcgttgc

SEQ ID NO: 363 - RNA, 21 nt, synthetic construct
  source 1..21: mol_type = other RNA
cgcgactactacatctccgtg

SEQ ID NO: 364 - RNA, 23 nt, synthetic construct
  source 1..23: mol_type = other RNA
cacggagatgtagtagtcgttgc

SEQ ID NO: 365 - RNA, 21 nt, synthetic construct
  source 1..21: mol_type = other RNA
cgcgactactacatctccgtg

SEQ ID NO: 366 - RNA, 23 nt, synthetic construct
  source 1..23: mol_type = other RNA
cacggagatgtagtagtcgttgc

SEQ ID NO: 367 - RNA, 19 nt, synthetic construct
  source 1..19: mol_type = other RNA
ttctccgaacgtgtcacgt

SEQ ID NO: 368 - RNA, 21 nt, synthetic construct
  source 1..21: mol_type = other RNA
acgtgacacgttcggagaact

SEQ ID NO: 369 - DNA, 20 bp, synthetic construct
  source 1..20: mol_type = other DNA
cagctgtgtgacgagtctgt

SEQ ID NO: 370 - DNA, 20 bp, synthetic construct
  source 1..20: mol_type = other DNA
ggcatccggggatcaaagat

SEQ ID NO: 371 - DNA, 19 bp, synthetic construct
  source 1..19: mol_type = other DNA
ggtcggagtcaacggattt

SEQ ID NO: 372 - DNA, 19 bp, synthetic construct
  source 1..19: mol_type = other DNA
ccagcatcgccccacttga

SEQ ID NO: 373 - RNA, 19 nt, synthetic construct
  source 1..19: mol_type = other RNA
ctgccatggagtatctgaa

SEQ ID NO: 374 - RNA, 21 nt, synthetic construct
  source 1..21: mol_type = other RNA
ttcagatactccatggcagtg

SEQ ID NO: 375 - RNA, 19 nt, synthetic construct
  source 1..19: mol_type = other RNA
ctgccatggagtatctgaa

SEQ ID NO: 376 - RNA, 21 nt, synthetic construct
  source 1..21: mol_type = other RNA
ttcagatactccatggcagtg

SEQ ID NO: 377 - RNA, 19 nt, synthetic construct
  source 1..19: mol_type = other RNA
acaacatcaagtactacga

SEQ ID NO: 378 - RNA, 21 nt, synthetic construct
  source 1..21: mol_type = other RNA
tcgtagtacttgatgttgttg

SEQ ID NO: 379 - RNA, 19 nt, synthetic construct
  source 1..19: mol_type = other RNA
acaacatcaagtactacga

SEQ ID NO: 380 - RNA, 21 nt, synthetic construct
  source 1..21: mol_type = other RNA
tcgtagtacttgatgttgttg

SEQ ID NO: 381 - RNA, 19 nt, synthetic construct
  source 1..19: mol_type = other RNA
cgactactacatctccgtg

SEQ ID NO: 382 - RNA, 21 nt, synthetic construct
  source 1..21: mol_type = other RNA
cacggagatgtagtagtcgtt

SEQ ID NO: 383 - RNA, 19 nt, synthetic construct
  source 1..19: mol_type = other RNA
cgactactacatctccgtg

SEQ ID NO: 384 - RNA, 21 nt, synthetic construct
  source 1..21: mol_type = other RNA
cacggagatgtagtagtcgtt